European Patent Specification EP 3 916 107 B1, published April 5, 2023. Title: MOLECULAR PROGRAMMING TOOLS. Applicant: President and Fellows of Harvard College. Application Not Yet Assigned. The sequence listing filed with the application follows.

SEQUENCE LISTING (7 sequences)

SEQ ID NO: 1 - DNA, 10 bp, Artificial Sequence
  Synthetic polynucleotide
atctcttatt

SEQ ID NO: 2 - DNA, 69 bp, Artificial Sequence
  Synthetic polynucleotide
  misc_feature (15)..(15): G is iisodG
  misc_feature (24)..(24): T is iBiodT
  misc_feature (32)..(32): Modified by a methyl group
  misc_feature (33)..(33): C is iMe-isodC
  misc_feature (60)..(60): C is iMe-isodC
  misc_feature (69)..(69): T is 3InvdT
acatactcatctcggcgctggtttttccagcgccgagatgagtatgtagttagagatgtcacgagatgt

SEQ ID NO: 3 - DNA, 69 bp, Artificial Sequence
  Synthetic  polynucleotide
  misc_feature (15)..(15): G is iisodG
  misc_feature (24)..(24): T is iBiodT
  misc_feature (32)..(32): Modified by a methyl group
  misc_feature (33)..(33): C is iMe-isodC
  misc_feature (69)..(69): T is 3InvdT
acatactcatctccgcgctggtttttccagcgcggagatgagtatgtagttagagatgtgacgagatgt

SEQ ID NO: 4 - DNA, 69 bp, Artificial Sequence
  Synthetic polynucleotide
  misc_feature (15)..(15): G is iisodG
  misc_feature (24)..(24): T is iBiodT
  misc_feature (32)..(32): Modified by a methyl group
  misc_feature (33)..(33): C is iMe-isodC
  misc_feature (59)..(59): Modified by a methyl group
  misc_feature (60)..(60): Modified by a methyl group
  misc_feature (61)..(61): Modified by a methyl group
  misc_feature (69)..(69): T is 3InvdT
acatactcatctcggcgctggtttttccagcgccgagatgagtatgtagttagagatgtgacgagatgt

SEQ ID NO: 5 - DNA, 10 bp, Artificial Sequence
  Synthetic polynucleotide
ttctcttatt

SEQ ID NO: 6 - DNA, 43 bp, Artificial Sequence
  Synthetic polynucleotide
actaaattcagggccttttggccctgaatttagtaataagaga

SEQ ID NO: 7 - DNA, 57 bp, Artificial Sequence
  Synthetic polynucleotide
ugugcaaaucuaugcaaaacugaatagtgggaggctagctacaacgagcggacattt